European Patent Application EP 4 556 022 A1, published May 21, 2025. Title: ANTI-NECTIN-4 ANTIBODY AND USE THEREOF. Applicant: Bio-Thera Solutions, Ltd. The sequence listing filed with the application follows.

SEQUENCE LISTING (368 sequences)

SEQ ID NO: 1 - protein, 18 aa, synthetic construct
MKWVTFISLLFLFSSAYS

SEQ ID NO: 2 - protein, 344 aa, synthetic construct
MKWVTFISLLFLFSSAYSGELETSDVVTVVLGQDAKLPCFYRGDSGEQVGQVAWARVDAGEGAQELALLHSKYGLHVSPAYEGRVEQPPPPRNPLDGSVLLRNAVQADEGEYECRVSTFPAGSFQARLRLRVLVPPLPSLNPGPALEEGQGLTLAASCTAEGSPAPSVTWDTEVKGTTSSRSFKHSRSAAVTSEFHLVPSRSMNGQPLTCVVSHPGLLQDQRITHILHVSFLAEASVRGLEDQNLWHIGREGAMLKCLSEGQPPPSYNWTRLDGPLPSGVRVDGDTLGFPPLTTEHSGIYVCHVSNEFSSRDSQVTVDVLDPQEDSGKQVDLVSASHHHHHHHH

SEQ ID NO: 3 - protein, 19 aa, synthetic construct
MELGLCWVFLVAILEGVQC

SEQ ID NO: 4 - protein, 22 aa, synthetic construct
MDMRVPAQLLGLLLLWFPGSRC

SEQ ID NO: 5 - protein, 447 aa, synthetic construct
EVQLVESGGGLVQPGGSLRLSCAASGFTFSSYNMNWVRQAPGKGLEWVSYISSSSSTIYYADSVKGRFTISRDNAKNSLSLQMNSLRDEDTAVYYCARAYYYGMDVWGQGTLVTVSSASTKGPSVFPLAPSSKSTSGGTAALGCLVKDYFPEPVTVSWNSGALTSGVHTFPAVLQSSGLYSLSSVVTVPSSSLGTQTYICNVNHKPSNTKVDKKVEPKSCDKTHTCPPCPAPELLGGPSVFLFPPKPKDTLMISRTPEVTCVVVDVSHEDPEVKFNWYVDGVEVHNAKTKPREEQYNSTYRVVSVLTVLHQDWLNGKEYKCKVSNKALPAPIEKTISKAKGQPREPQVYTLPPSRDELTKNQVSLTCLVKGFYPSDIAVEWESNGQPENNYKTTPPVLDSDGSFFLYSKLTVDKSRWQQGNVFSCSVMHEALHNHYTQKSLSLSPGK

SEQ ID NO: 6 - protein, 214 aa, synthetic construct
DIQMTQSPSSVSASVGDRVTITCRASQGISGWLAWYQQKPGKAPKFLIYAASTLQSGVPSRFSGSGSGTDFTLTISSLQPEDFATYYCQQANSFPPTFGGGTKVEIKRTVAAPSVFIFPPSDEQLKSGTASVVCLLNNFYPREAKVQWKVDNALQSGNSQESVTEQDSKDSTYSLSSTLTLSKADYEKHKVYACEVTHQGLSSPVTKSFNRGEC

SEQ ID NO: 7 - protein, 122 aa, synthetic construct
EVQLVESGGGLVQPGGSLRLSCAASGFTFSSYAMSWVRQAPGKGLEWVSAISGSGGSTYYADSVKGRFTISRDNSKNTLYLQMNSLRAEDTAVYYCARQTEDRYYGYDLDYWGQGTLVTVSS

SEQ ID NO: 8 - protein, 5 aa, synthetic construct
SYAMS

SEQ ID NO: 9 - protein, 17 aa, synthetic construct
AISGSGGSTYYADSVKG

SEQ ID NO: 10 - protein, 13 aa, synthetic construct
QTEDRYYGYDLDY

SEQ ID NO: 11 - protein, 122 aa, synthetic construct
EVQLVESGGGLVQPGGSLRLSCAASGFTFSSYAMSWVRQAPGKGLEWVSAISGSGGSTYYADSVKGRFTISRDNSKNTLYLQMNSLRAEDTAVYYCARQTEDRSYGYDLDYWGQGTLVTVSS

SEQ ID NO: 12 - protein, 13 aa, synthetic construct
QTEDRSYGYDLDY

SEQ ID NO: 13 - protein, 123 aa, synthetic construct
EVQLVESGGGLVQPGGSLRLSCAASGFTFSSYAMSWVRQAPGKGLEWVSAISGSGGSTYYADSVKGRFTISRDNSKNTLYLQMNSLRAEDTAVYYCARAELLAFDVYTASDYWGQGTLVTVSS

SEQ ID NO: 14 - protein, 14 aa, synthetic construct
AELLAFDVYTASDY

SEQ ID NO: 15 - protein, 126 aa, synthetic construct
EVQLVESGGGLVQPGGSLRLSCAASGFTFSSYAMSWVRQAPGKGLEWVSAISGSGGSTYYADSVKGRFTISRDNSKNTLYLQMNSLRAEDTAVYYCAREYSDVVDYVSVRTPLDYWGQGTLVTVSS

SEQ ID NO: 16 - protein, 17 aa, synthetic construct
EYSDVVDYVSVRTPLDY

SEQ ID NO: 17 - protein, 126 aa, synthetic construct
EVQLVESGGGLVQPGGSLRLSCAASGFTFSSYAMSWVRQAPGKGLEWVSAISGSGGSTYYADSVKGRFTISRDNSKNTLYLQMNSLRAEDTAVYYCARDRSDVYSYSYFPTPLDYWGQGTLVTVSS

SEQ ID NO: 18 - protein, 17 aa, synthetic construct
DRSDVYSYSYFPTPLDY

SEQ ID NO: 19 - protein, 122 aa, synthetic construct
EVQLVESGGGLVQPGGSLRLSCAASGFTFSSYAMSWVRQAPGKGLEWVSAISGSGGSTYYADSVKGRFTISRDNSKNTLYLQMNSLRAEDTAVYYCARQTEDRSYGYDMDYWGQGTLVTVSS

SEQ ID NO: 20 - protein, 13 aa, synthetic construct
QTEDRSYGYDMDY

SEQ ID NO: 21 - protein, 123 aa, synthetic construct
EVQLVESGGGLVQPGGSLRLSCAASGFTFSSYAMSWVRQAPGKGLEWVSAISGSGGSTYYADSVKGRFTISRDNSKNTLYLQMNSLRAEDTAVYYCARERSDATYLRTPLDYWGQGTLVTVSS

SEQ ID NO: 22 - protein, 14 aa, synthetic construct
ERSDATYLRTPLDY

SEQ ID NO: 23 - protein, 122 aa, synthetic construct
EVQLVESGGGLVQPGGSLRLSCAASGFTFSSYAMSWVRQAPGKGLEWVSAISGSGGSTYYADSVKGRFTISRDNSKNTLYLQMNSLRAEDTAVYYCARHTEDRYYGYYLDYWGQGTLVTVSS

SEQ ID NO: 24 - protein, 13 aa, synthetic construct
HTEDRYYGYYLDY

SEQ ID NO: 25 - protein, 108 aa, synthetic construct
DIQMTQSPSSLSASVGDRVTITCRASQGISSYLAWYQQKPGKAPKLLIYAASSLQSGVPSRFSGSGSGTDFTLTISSLQPEDFATYYCQQHYTTPPTFGQGTKVEIKR

SEQ ID NO: 26 - protein, 11 aa, synthetic construct
RASQGISSYLA

SEQ ID NO: 27 - protein, 7 aa, synthetic construct
AASSLQS

SEQ ID NO: 28 - protein, 9 aa, synthetic construct
QQHYTTPPT

SEQ ID NO: 29 - protein, 30 aa, synthetic construct
EVQLVESGGGLVQPGGSLRLSCAASGFTFS

SEQ ID NO: 30 - protein, 14 aa, synthetic construct
WVRQAPGKGLEWVS

SEQ ID NO: 31 - protein, 32 aa, synthetic construct
RFTISRDNSKNTLYLQMNSLRAEDTAVYYCAR

SEQ ID NO: 32 - protein, 11 aa, synthetic construct
WGQGTLVTVSS

SEQ ID NO: 33 - protein, 23 aa, synthetic construct
DIQMTQSPSSLSASVGDRVTITC

SEQ ID NO: 34 - protein, 15 aa, synthetic construct
WYQQKPGKAPKLLIY

SEQ ID NO: 35 - protein, 32 aa, synthetic construct
GVPSRFSGSGSGTDFTLTISSLQPEDFATYYC

SEQ ID NO: 36 - protein, 11 aa, synthetic construct
FGQGTKVEIKR

SEQ ID NO: 37 - protein, 330 aa, synthetic construct [sequence omitted]

SEQ ID NO: 38 - protein, 106 aa, synthetic construct
TVAAPSVFIFPPSDEQLKSGTASVVCLLNNFYPREAKVQWKVDNALQSGNSQESVTEQDSKDSTYSLSSTLTLSKADYEKHKVYACEVTHQGLSSPVTKSFNRGEC

SEQ ID NO: 39 - protein, 19 aa, synthetic construct
MEWSWVFLFFLSVTTGVHS

SEQ ID NO: 40 - protein, 22 aa, synthetic construct
MDMRVPAQLLGLLLLWLPGARC

SEQ ID NO: 41 - protein, 123 aa, synthetic construct
EVQLVESGGGLVQPGGSLRLSCAASGYSFDNYAMSWVRQAPGKGLEWVSRISPTGGYASYADSVKGRFTISRDNSKNTLYLQMNSLRAEDTAVYYCARAELLAFDVYTASDYWGQGTLVTVSS

SEQ ID NO: 42 - protein, 123 aa, synthetic construct
EVQLVESGGGLVQPGGSLRLSCAASGFTFGTYGMSWVRQAPGKGLEWVSGIKPGDSTTYYADSVKGRFTISRDNSKNTLYLQMNSLRAEDTAVYYCARAELLAFDVYTASDYWGQGTLVTVSS

SEQ ID NO: 43 - protein, 123 aa, synthetic construct
EVQLVESGGGLVQPGGSLRLSCAASGFNFSSYGMSWVRQAPGKGLEWVSAISGSGGSTYYADSVKGRFTISRDNSKNTLYLQMNSLRAEDTAVYYCARAELLAFDVYTASDYWGQGTLVTVSS

SEQ ID NO: 44 - protein, 123 aa, synthetic construct
EVQLVESGGGLVQPGGSLRLSCAASGFTFGDYGMSWVRQAPGKGLEWVSGIKPWGSGTYYADSVKGRFTISRDNSKNTLYLQMNSLRAEDTAVYYCARAELLAFDVYTASDYWGQGTLVTVSS

SEQ ID NO: 45 - protein, 123 aa, synthetic construct
EVQLVESGGGLVQPGGSLRLSCAASGDIFTNYSMSWVRQAPGKGLEWVSGIYPSGDNNRYADSVKGRFTISRDNSKNTLYLQMNSLRAEDTAVYYCARAELLAFDVYTASDYWGQGTLVTVSS

SEQ ID NO: 46 - protein, 123 aa, synthetic construct
EVQLVESGGGLVQPGGSLRLSCAASGYNFTDYGMSWVRQAPGKGLEWVSGISGSGDNKYYADSVKGRFTISRDNSKNTLYLQMNSLRAEDTAVYYCARAELLAFDVYTASDYWGQGTLVTVSS

SEQ ID NO: 47 - protein, 123 aa, synthetic construct
EVQLVESGGGLVQPGGSLRLSCAASGGSFYGFGMSWVRQAPGKGLEWVSGIYSHDADKRYADSVKGRFTISRDNSKNTLYLQMNSLRAEDTAVYYCARAELLAFDVYTASDYWGQGTLVTVSS

SEQ ID NO: 48 - protein, 123 aa, synthetic construct
EVQLVESGGGLVQPGGSLRLSCAASGFSFDDYAMSWVRQAPGKGLEWVSIIYPTGSTNYYADSVKGRFTISRDNSKNTLYLQMNSLRAEDTAVYYCARAELLAFDVYTASDYWGQGTLVTVSS

SEQ ID NO: 49 - protein, 123 aa, synthetic construct
EVQLVESGGGLVQPGGSLRLSCAASGFNFSSYGMSWVRQAPGKGLEWVSRISPYTDNKYYADSVKGRFTISRDNSKNTLYLQMNSLRAEDTAVYYCARAELLAFDVYTASDYWGQGTLVTVSS

SEQ ID NO: 50 - protein, 123 aa, synthetic construct
EVQLVESGGGLVQPGGSLRLSCAASGFSFGTYGMSWVRQAPGKGLEWVSRISGDSANIRYADSVKGRFTISRDNSKNTLYLQMNSLRAEDTAVYYCARAELLAFDVYTASDYWGQGTLVTVSS

SEQ ID NO: 51 - protein, 123 aa, synthetic construct
EVQLVESGGGLVQPGGSLRLSCAASGFTFDDYAMSWVRQAPGKGLEWVSGIKPSSWTTYYADSVKGRFTISRDNSKNTLYLQMNSLRAEDTAVYYCARAELLAFDVYTASDYWGQGTLVTVSS

SEQ ID NO: 52 - protein, 123 aa, synthetic construct
EVQLVESGGGLVQPGGSLRLSCAASGDIFTGSSMSWVRQAPGKGLEWVSGIYASGSDKRYADSVKGRFTISRDNSKNTLYLQMNSLRAEDTAVYYCARAELLAFDVYTASDYWGQGTLVTVSS

SEQ ID NO: 53 - protein, 123 aa, synthetic construct
EVQLVESGGGLVQPGGSLRLSCAASGFNFGNYGMSWVRQAPGKGLEWVSRISGDGSNINYADSVKGRFTISRDNSKNTLYLQMNSLRAEDTAVYYCARAELLAFDVYTASDYWGQGTLVTVSS

SEQ ID NO: 54 - protein, 123 aa, synthetic construct
EVQLVESGGGLVQPGGSLRLSCAASGYSFTGYGMSWVRQAPGKGLEWVSGISPSGGTIGYADSVKGRFTISRDNSKNTLYLQMNSLRAEDTAVYYCARAELLAFDVYTASDYWGQGTLVTVSS

SEQ ID NO: 55 - protein, 123 aa, synthetic construct
EVQLVESGGGLVQPGGSLRLSCAASGYTFGDYGMSWVRQAPGKGLEWVSRIDPWGASIRYADSVKGRFTISRDNSKNTLYLQMNSLRAEDTAVYYCARAELLAFDVYTASDYWGQGTLVTVSS

SEQ ID NO: 56 - protein, 123 aa, synthetic construct
EVQLVESGGGLVQPGGSLRLSCAASGFSFGSYGMSWVRQAPGKGLEWVSGIKPSTSTTYYADSVKGRFTISRDNSKNTLYLQMNSLRAEDTAVYYCARAELLAFDVYTASDYWGQGTLVTVSS

SEQ ID NO: 57 - protein, 123 aa, synthetic construct
EVQLVESGGGLVQPGGSLRLSCAASGDIFSNYSMSWVRQAPGKGLEWVSGIYPSGDSRRYADSVKGRFTISRDNSKNTLYLQMNSLRAEDTAVYYCARAELLAFDVYTASDYWGQGTLVTVSS

SEQ ID NO: 58 - protein, 123 aa, synthetic construct
EVQLVESGGGLVQPGGSLRLSCAASGFNFTDYGMSWVRQAPGKGLEWVSRISQWGDTSNYADSVKGRFTISRDNSKNTLYLQMNSLRAEDTAVYYCARAELLAFDVYTASDYWGQGTLVTVSS

SEQ ID NO: 59 - protein, 123 aa, synthetic construct
EVQLVESGGGLVQPGGSLRLSCAASGFNFYNYGMSWVRQAPGKGLEWVSGIKPHSDVAHYADSVKGRFTISRDNSKNTLYLQMNSLRAEDTAVYYCARAELLAFDVYTASDYWGQGTLVTVSS

SEQ ID NO: 60 - protein, 123 aa, synthetic construct
EVQLVESGGGLVQPGGSLRLSCAASGDNFYTFYMSWVRQAPGKGLEWVSGIKPTGSYINYADSVKGRFTISRDNSKNTLYLQMNSLRAEDTAVYYCARAELLAFDVYTASDYWGQGTLVTVSS

SEQ ID NO: 61 - protein, 123 aa, synthetic construct
EVQLVESGGGLVQPGGSLRLSCAASGYSFDSYGMSWVRQAPGKGLEWVSGIKPTGASTYYADSVKGRFTISRDNSKNTLYLQMNSLRAEDTAVYYCARAELLAFDVYTASDYWGQGTLVTVSS

SEQ ID NO: 62 - protein, 123 aa, synthetic construct
EVQLVESGGGLVQPGGSLRLSCAASGYNFDNYAMSWVRQAPGKGLEWVSGIKPDSATTYYADSVKGRFTISRDNSKNTLYLQMNSLRAEDTAVYYCARAELLAFDVYTASDYWGQGTLVTVSS

SEQ ID NO: 63 - protein, 123 aa, synthetic construct
EVQLVESGGGLVQPGGSLRLSCAASGYNFYSYGMSWVRQAPGKGLEWVSIISPDGGYKRYADSVKGRFTISRDNSKNTLYLQMNSLRAEDTAVYYCARAELLAFDVYTASDYWGQGTLVTVSS

SEQ ID NO: 64 - protein, 123 aa, synthetic construct
EVQLVESGGGLVQPGGSLRLSCAASGYSFSDFGMSWVRQAPGKGLEWVSRIDPSGWSTSYADSVKGRFTISRDNSKNTLYLQMNSLRAEDTAVYYCARAELLAFDVYTASDYWGQGTLVTVSS

SEQ ID NO: 65 - protein, 123 aa, synthetic construct
EVQLVESGGGLVQPGGSLRLSCAASGFNFDSYAMSWVRQAPGKGLEWVSGIKPHTDDIYYADSVKGRFTISRDNSKNTLYLQMNSLRAEDTAVYYCARAELLAFDVYTASDYWGQGTLVTVSS

SEQ ID NO: 66 - protein, 123 aa, synthetic construct
EVQLVESGGGLVQPGGSLRLSCAASGDIFTNYSMSWVRQAPGKGLEWVSGIYASGSDKRYADSVKGRFTISRDNSKNTLYLQMNSLRAEDTAVYYCARAELLAFDVYTASDYWGQGTLVTVSS

SEQ ID NO: 67 - protein, 123 aa, synthetic construct
EVQLVESGGGLVQPGGSLRLSCAASGFNFGGYGMSWVRQAPGKGLEWVSRISPGDSTPRYADSVKGRFTISRDNSKNTLYLQMNSLRAEDTAVYYCARAELLAFDVYTASDYWGQGTLVTVSS

SEQ ID NO: 68 - protein, 123 aa, synthetic construct
EVQLVESGGGLVQPGGSLRLSCAASGFNFSSYGMSWVRQAPGKGLEWVSRISPYTGTTHYADSVKGRFTISRDNSKNTLYLQMNSLRAEDTAVYYCARAELLAFDVYTASDYWGQGTLVTVSS

SEQ ID NO: 69 - protein, 123 aa, synthetic construct
EVQLVESGGGLVQPGGSLRLSCAASGYSFSDYGMSWVRQAPGKGLEWVSRISPSKAVKDYADSVKGRFTISRDNSKNTLYLQMNSLRAEDTAVYYCARAELLAFDVYTASDYWGQGTLVTVSS

SEQ ID NO: 70 - protein, 123 aa, synthetic construct
EVQLVESGGGLVQPGGSLRLSCAASGGNFTNSGMSWVRQAPGKGLEWVSGIKWSSDETYYADSVKGRFTISRDNSKNTLYLQMNSLRAEDTAVYYCARAELLAFDVYTASDYWGQGTLVTVSS

SEQ ID NO: 71 - protein, 123 aa, synthetic construct
EVQLVESGGGLVQPGGSLRLSCAASGYSFSDYGMSWVRQAPGKGLEWVSWISPSKGSASYADSVKGRFTISRDNSKNTLYLQMNSLRAEDTAVYYCARAELLAFDVYTASDYWGQGTLVTVSS

SEQ ID NO: 72 - protein, 123 aa, synthetic construct
EVQLVESGGGLVQPGGSLRLSCAASGDIFTGYSMSWVRQAPGKGLEWVSGIYQTGSNTRYADSVKGRFTISRDNSKNTLYLQMNSLRAEDTAVYYCARAELLAFDVYTASDYWGQGTLVTVSS

SEQ ID NO: 73 - protein, 123 aa, synthetic construct
EVQLVESGGGLVQPGGSLRLSCAASGFNFSDYGMSWVRQAPGKGLEWVSRIDWDGGNTRYADSVKGRFTISRDNSKNTLYLQMNSLRAEDTAVYYCARAELLAFDVYTASDYWGQGTLVTVSS

SEQ ID NO: 74 - protein, 123 aa, synthetic construct
EVQLVESGGGLVQPGGSLRLSCAASGFTFSDYGMSWVRQAPGKGLEWVSRISQYGGGIRYADSVKGRFTISRDNSKNTLYLQMNSLRAEDTAVYYCARAELLAFDVYTASDYWGQGTLVTVSS

SEQ ID NO: 75 - protein, 123 aa, synthetic construct
EVQLVESGGGLVQPGGSLRLSCAASGFNFSNYGMSWVRQAPGKGLEWVSRIKPTDGSTHYADSVKGRFTISRDNSKNTLYLQMNSLRAEDTAVYYCARAELLAFDVYTASDYWGQGTLVTVSS

SEQ ID NO: 76 - protein, 123 aa, synthetic construct
EVQLVESGGGLVQPGGSLRLSCAASGFTFGGYGMSWVRQAPGKGLEWVSWISAWDGSIYYADSVKGRFTISRDNSKNTLYLQMNSLRAEDTAVYYCARAELLAFDVYTASDYWGQGTLVTVSS

SEQ ID NO: 77 - protein, 123 aa, synthetic construct
EVQLVESGGGLVQPGGSLRLSCAASGDSFDSSGMSWVRQAPGKGLEWVSGIKWITGESYYADSVKGRFTISRDNSKNTLYLQMNSLRAEDTAVYYCARAELLAFDVYTASDYWGQGTLVTVSS

SEQ ID NO: 78 - protein, 123 aa, synthetic construct
EVQLVESGGGLVQPGGSLRLSCAASGYTFSSYGMSWVRQAPGKGLEWVSRIKSDGGDTHYADSVKGRFTISRDNSKNTLYLQMNSLRAEDTAVYYCARAELLAFDVYTASDYWGQGTLVTVSS

SEQ ID NO: 79 - protein, 122 aa, synthetic construct
EVQLVESGGGLVQPGGSLRLSCAASGGTFDTNAMSWVRQAPGKGLEWVSAISTGGDNKRYADSVKGRFTISRDNSKNTLYLQMNSLRAEDTAVYYCARQTEDRSYGYDLDYWGQGTLVTVSS

SEQ ID NO: 80 - protein, 122 aa, synthetic construct
EVQLVESGGGLVQPGGSLRLSCAASGYNFGSYAMSWVRQAPGKGLEWVSRIYPGSWSPDYADSVKGRFTISRDNSKNTLYLQMNSLRAEDTAVYYCARQTEDRSYGYDLDYWGQGTLVTVSS

SEQ ID NO: 81 - protein, 122 aa, synthetic construct
EVQLVESGGGLVQPGGSLRLSCAASGYTFDSYAMSWVRQAPGKGLEWVSRIKTTDDGKSYADSVKGRFTISRDNSKNTLYLQMNSLRAEDTAVYYCARQTEDRSYGYDLDYWGQGTLVTVSS

SEQ ID NO: 82 - protein, 122 aa, synthetic construct
EVQLVESGGGLVQPGGSLRLSCAASGYNFSNYAMSWVRQAPGKGLEWVSAIDASGGDTRYADSVKGRFTISRDNSKNTLYLQMNSLRAEDTAVYYCARQTEDRSYGYDLDYWGQGTLVTVSS

SEQ ID NO: 83 - protein, 122 aa, synthetic construct
EVQLVESGGGLVQPGGSLRLSCAASGYSFSNYAMSWVRQAPGKGLEWVSRISAWGSTNNYADSVKGRFTISRDNSKNTLYLQMNSLRAEDTAVYYCARQTEDRSYGYDLDYWGQGTLVTVSS

SEQ ID NO: 84 - protein, 122 aa, synthetic construct
EVQLVESGGGLVQPGGSLRLSCAASGYIFSNYAMSWVRQAPGKGLEWVSRISTGFAGPDYADSVKGRFTISRDNSKNTLYLQMNSLRAEDTAVYYCARQTEDRSYGYDLDYWGQGTLVTVSS

SEQ ID NO: 85 - protein, 122 aa, synthetic construct
EVQLVESGGGLVQPGGSLRLSCAASGFNFSDYSMSWVRQAPGKGLEWVSRIKASSGGSDYADSVKGRFTISRDNSKNTLYLQMNSLRAEDTAVYYCARQTEDRSYGYDLDYWGQGTLVTVSS

SEQ ID NO: 86 - protein, 122 aa, synthetic construct
EVQLVESGGGLVQPGGSLRLSCAASGGSFYGFGMSWVRQAPGKGLEWVSGIYSHDADKRYADSVKGRFTISRDNSKNTLYLQMNSLRAEDTAVYYCARQTEDRSYGYDLDYWGQGTLVTVSS

SEQ ID NO: 87 - protein, 122 aa, synthetic construct
EVQLVESGGGLVQPGGSLRLSCAASGFSFGSSAMSWVRQAPGKGLEWVSAISGSSDSPRYADSVKGRFTISRDNSKNTLYLQMNSLRAEDTAVYYCARQTEDRSYGYDLDYWGQGTLVTVSS

SEQ ID NO: 88 - protein, 122 aa, synthetic construct
EVQLVESGGGLVQPGGSLRLSCAASGDIFTGYAMSWVRQAPGKGLEWVSRIDGTGDSKFYADSVKGRFTISRDNSKNTLYLQMNSLRAEDTAVYYCARQTEDRSYGYDLDYWGQGTLVTVSS

SEQ ID NO: 89 - protein, 122 aa, synthetic construct
EVQLVESGGGLVQPGGSLRLSCAASGGSFSNYAMSWVRQAPGKGLEWVSWIDTTSAYASYADSVKGRFTISRDNSKNTLYLQMNSLRAEDTAVYYCARQTEDRSYGYDLDYWGQGTLVTVSS

SEQ ID NO: 90 - protein, 122 aa, synthetic construct
EVQLVESGGGLVQPGGSLRLSCAASGDSFSTYAMSWVRQAPGKGLEWVSRISGSGDGKDYADSVKGRFTISRDNSKNTLYLQMNSLRAEDTAVYYCARQTEDRSYGYDLDYWGQGTLVTVSS

SEQ ID NO: 91 - protein, 122 aa, synthetic construct
EVQLVESGGGLVQPGGSLRLSCAASGFNFTSYAMSWVRQAPGKGLEWVSRISAHKWDASYADSVKGRFTISRDNSKNTLYLQMNSLRAEDTAVYYCARQTEDRSYGYDLDYWGQGTLVTVSS

SEQ ID NO: 92 - protein, 122 aa, synthetic construct
EVQLVESGGGLVQPGGSLRLSCAASGYIFTDYSMSWVRQAPGKGLEWVSRIYTDGWEKDYADSVKGRFTISRDNSKNTLYLQMNSLRAEDTAVYYCARQTEDRSYGYDLDYWGQGTLVTVSS

SEQ ID NO: 93 - protein, 122 aa, synthetic construct
EVQLVESGGGLVQPGGSLRLSCAASGFTFDGYAMSWVRQAPGKGLEWVSRISSYSWNPDYADSVKGRFTISRDNSKNTLYLQMNSLRAEDTAVYYCARQTEDRSYGYDLDYWGQGTLVTVSS

SEQ ID NO: 94 - protein, 122 aa, synthetic construct
EVQLVESGGGLVQPGGSLRLSCAASGDTFSSYAMSWVRQAPGKGLEWVSRISQTGGTTDYADSVKGRFTISRDNSKNTLYLQMNSLRAEDTAVYYCARQTEDRSYGYDLDYWGQGTLVTVSS

SEQ ID NO: 95 - protein, 120 aa, synthetic construct
EVQLVESGGGLVQPGGSLRLSCAASGDIFDTYMSWVRQAPGKGLEWVSRIYTDGSSDYADSVKGRFTISRDNSKNTLYLQMNSLRAEDTAVYYCARQTEDRSYGYDLDYWGQGTLVTVSS

SEQ ID NO: 96 - protein, 122 aa, synthetic construct
EVQLVESGGGLVQPGGSLRLSCAASGYSFYGYAMSWVRQAPGKGLEWVSAIDAIGGNKRYADSVKGRFTISRDNSKNTLYLQMNSLRAEDTAVYYCARQTEDRSYGYDLDYWGQGTLVTVSS

SEQ ID NO: 97 - protein, 122 aa, synthetic construct
EVQLVESGGGLVQPGGSLRLSCAASGYNFTSSAMSWVRQAPGKGLEWVSRIYSISGNTDYADSVKGRFTISRDNSKNTLYLQMNSLRAEDTAVYYCARQTEDRSYGYDLDYWGQGTLVTVSS

SEQ ID NO: 98 - protein, 122 aa, synthetic construct
EVQLVESGGGLVQPGGSLRLSCAASGFNFGTYAMSWVRQAPGKGLEWVSRISGISAGTNYADSVKGRFTISRDNSKNTLYLQMNSLRAEDTAVYYCARQTEDRSYGYDLDYWGQGTLVTVSS

SEQ ID NO: 99 - protein, 122 aa, synthetic construct
EVQLVESGGGLVQPGGSLRLSCAASGYNFTTSAMSWVRQAPGKGLEWVSRIYADTAYNDYADSVKGRFTISRDNSKNTLYLQMNSLRAEDTAVYYCARQTEDRSYGYDLDYWGQGTLVTVSS

SEQ ID NO: 100 - protein, 122 aa, synthetic construct
EVQLVESGGGLVQPGGSLRLSCAASGFNFGDFAMSWVRQAPGKGLEWVSRIYSGDDNASYADSVKGRFTISRDNSKNTLYLQMNSLRAEDTAVYYCARQTEDRSYGYDLDYWGQGTLVTVSS

SEQ ID NO: 101 - protein, 122 aa, synthetic construct
EVQLVESGGGLVQPGGSLRLSCAASGDTFSGYAMSWVRQAPGKGLEWVSRIYPYSSVRDYADSVKGRFTISRDNSKNTLYLQMNSLRAEDTAVYYCARQTEDRSYGYDLDYWGQGTLVTVSS

SEQ ID NO: 102 - protein, 122 aa, synthetic construct
EVQLVESGGGLVQPGGSLRLSCAASGFNFSGFAMSWVRQAPGKGLEWVSRIYPTSSESDYADSVKGRFTISRDNSKNTLYLQMNSLRAEDTAVYYCARQTEDRSYGYDLDYWGQGTLVTVSS

SEQ ID NO: 103 - protein, 122 aa, synthetic construct
EVQLVESGGGLVQPGGSLRLSCAASGYSFDGFAMSWVRQAPGKGLEWVSRISGHDWSSSYADSVKGRFTISRDNSKNTLYLQMNSLRAEDTAVYYCARQTEDRSYGYDLDYWGQGTLVTVSS

SEQ ID NO: 104 - protein, 122 aa, synthetic construct
EVQLVESGGGLVQPGGSLRLSCAASGDSFYNYSMSWVRQAPGKGLEWVSRISSDGWETFYADSVKGRFTISRDNSKNTLYLQMNSLRAEDTAVYYCARQTEDRSYGYDLDYWGQGTLVTVSS

SEQ ID NO: 105 - protein, 122 aa, synthetic construct
EVQLVESGGGLVQPGGSLRLSCAASGDTFSSNAMSWVRQAPGKGLEWVSRIYGGSWDTDYADSVKGRFTISRDNSKNTLYLQMNSLRAEDTAVYYCARQTEDRSYGYDLDYWGQGTLVTVSS

SEQ ID NO: 106 - protein, 122 aa, synthetic construct
EVQLVESGGGLVQPGGSLRLSCAASGYSFSDYAMSWVRQAPGKGLEWVSRISAYGWGKSYADSVKGRFTISRDNSKNTLYLQMNSLRAEDTAVYYCARQTEDRSYGYDLDYWGQGTLVTVSS

SEQ ID NO: 107 - protein, 122 aa, synthetic construct
EVQLVESGGGLVQPGGSLRLSCAASGFSFTNNAMSWVRQAPGKGLEWVSRIDTIGGTSSYADSVKGRFTISRDNSKNTLYLQMNSLRAEDTAVYYCARQTEDRSYGYDLDYWGQGTLVTVSS

SEQ ID NO: 108 - protein, 122 aa, synthetic construct
EVQLVESGGGLVQPGGSLRLSCAASGDTFGTSSMSWVRQAPGKGLEWVSRIDTWGWYKFYADSVKGRFTISRDNSKNTLYLQMNSLRAEDTAVYYCARQTEDRSYGYDLDYWGQGTLVTVSS

SEQ ID NO: 109 - protein, 122 aa, synthetic construct
EVQLVESGGGLVQPGGSLRLSCAASGYNFTTSAMSWVRQAPGKGLEWVSRIYQDSSTTDYADSVKGRFTISRDNSKNTLYLQMNSLRAEDTAVYYCARQTEDRSYGYDLDYWGQGTLVTVSS

SEQ ID NO: 110 - protein, 122 aa, synthetic construct
EVQLVESGGGLVQPGGSLRLSCAASGYNFGNYAMSWVRQAPGKGLEWVSRIKSHDSTSHYADSVKGRFTISRDNSKNTLYLQMNSLRAEDTAVYYCARQTEDRSYGYDLDYWGQGTLVTVSS

SEQ ID NO: 111 - protein, 122 aa, synthetic construct
EVQLVESGGGLVQPGGSLRLSCAASGGSFGGYAMSWVRQAPGKGLEWVSRIYAYKSENDYADSVKGRFTISRDNSKNTLYLQMNSLRAEDTAVYYCARQTEDRSYGYDLDYWGQGTLVTVSS

SEQ ID NO: 112 - protein, 122 aa, synthetic construct
EVQLVESGGGLVQPGGSLRLSCAASGDNFSSYAMSWVRQAPGKGLEWVSRIYGSDSTPDYADSVKGRFTISRDNSKNTLYLQMNSLRAEDTAVYYCARQTEDRSYGYDLDYWGQGTLVTVSS

SEQ ID NO: 113 - protein, 122 aa, synthetic construct
EVQLVESGGGLVQPGGSLRLSCAASGYSFTNFAMSWVRQAPGKGLEWVSRISQDGGNKNYADSVKGRFTISRDNSKNTLYLQMNSLRAEDTAVYYCARQTEDRSYGYDLDYWGQGTLVTVSS

SEQ ID NO: 114 - protein, 122 aa, synthetic construct
EVQLVESGGGLVQPGGSLRLSCAASGYSFSGNAMSWVRQAPGKGLEWVSRIDGWGSYTDYADSVKGRFTISRDNSKNTLYLQMNSLRAEDTAVYYCARQTEDRSYGYDLDYWGQGTLVTVSS

SEQ ID NO: 115 - protein, 122 aa, synthetic construct
EVQLVESGGGLVQPGGSLRLSCAASGYNFGGYAMSWVRQAPGKGLEWVSRISGTSGNNDYADSVKGRFTISRDNSKNTLYLQMNSLRAEDTAVYYCARQTEDRSYGYDLDYWGQGTLVTVSS

SEQ ID NO: 116 - protein, 122 aa, synthetic construct
EVQLVESGGGLVQPGGSLRLSCAASGFSFDGYAMSWVRQAPGKGLEWVSRISAHSWNKDYADSVKGRFTISRDNSKNTLYLQMNSLRAEDTAVYYCARQTEDRSYGYDLDYWGQGTLVTVSS

SEQ ID NO: 117 - protein, 122 aa, synthetic construct
EVQLVESGGGLVQPGGSLRLSCAASGDSFTSYAMSWVRQAPGKGLEWVSRISADSASPSYADSVKGRFTISRDNSKNTLYLQMNSLRAEDTAVYYCARQTEDRSYGYDLDYWGQGTLVTVSS

SEQ ID NO: 118 - protein, 122 aa, synthetic construct
EVQLVESGGGLVQPGGSLRLSCAASGDIFDGYSMSWVRQAPGKGLEWVSRIDTGGSVKNYADSVKGRFTISRDNSKNTLYLQMNSLRAEDTAVYYCARQTEDRSYGYDLDYWGQGTLVTVSS

SEQ ID NO: 119 - protein, 122 aa, synthetic construct
EVQLVESGGGLVQPGGSLRLSCAASGYTFGNYAMSWVRQAPGKGLEWVSRISPSTWNIDYADSVKGRFTISRDNSKNTLYLQMNSLRAEDTAVYYCARQTEDRSYGYDLDYWGQGTLVTVSS

SEQ ID NO: 120 - protein, 122 aa, synthetic construct
EVQLVESGGGLVQPGGSLRLSCAASGYTFGSNAMSWVRQAPGKGLEWVSRISPDSSGISYADSVKGRFTISRDNSKNTLYLQMNSLRAEDTAVYYCARQTEDRSYGYDLDYWGQGTLVTVSS

SEQ ID NO: 121 - protein, 122 aa, synthetic construct
EVQLVESGGGLVQPGGSLRLSCAASGDIFGSYAMSWVRQAPGKGLEWVSRISSHGASRDYADSVKGRFTISRDNSKNTLYLQMNSLRAEDTAVYYCARQTEDRSYGYDLDYWGQGTLVTVSS

SEQ ID NO: 122 - protein, 122 aa, synthetic construct; identical to SEQ ID NO: 83

SEQ ID NO: 123 - protein, 122 aa, synthetic construct
EVQLVESGGGLVQPGGSLRLSCAASGFTFSNNAMSWVRQAPGKGLEWVSAIYASTDGRSYADSVKGRFTISRDNSKNTLYLQMNSLRAEDTAVYYCARQTEDRSYGYDLDYWGQGTLVTVSS

SEQ ID NO: 124 - protein, 122 aa, synthetic construct
EVQLVESGGGLVQPGGSLRLSCAASGFIFGGNAMSWVRQAPGKGLEWVSRISSDKGTTNYADSVKGRFTISRDNSKNTLYLQMNSLRAEDTAVYYCARQTEDRSYGYDLDYWGQGTLVTVSS

SEQ ID NO: 125 - protein, 122 aa, synthetic construct
EVQLVESGGGLVQPGGSLRLSCAASGFTFGGYSMSWVRQAPGKGLEWVSRISTDGAYTNYADSVKGRFTISRDNSKNTLYLQMNSLRAEDTAVYYCARQTEDRSYGYDLDYWGQGTLVTVSS

SEQ ID NO: 126 - protein, 122 aa, synthetic construct
EVQLVESGGGLVQPGGSLRLSCAASGGTFYTYAMSWVRQAPGKGLEWVSRIYSTKGTPDYADSVKGRFTISRDNSKNTLYLQMNSLRAEDTAVYYCARQTEDRSYGYDLDYWGQGTLVTVSS

SEQ ID NO: 127 - protein, 122 aa, synthetic construct
EVQLVESGGGLVQPGGSLRLSCAASGFNFTNYAMSWVRQAPGKGLEWVSRISTYGDTTHYADSVKGRFTISRDNSKNTLYLQMNSLRAEDTAVYYCARQTEDRSYGYDLDYWGQGTLVTVSS

SEQ ID NO: 128 - protein, 122 aa, synthetic construct
EVQLVESGGGLVQPGGSLRLSCAASGYIFTNYAMSWVRQAPGKGLEWVSRISQSGGTNDYADSVKGRFTISRDNSKNTLYLQMNSLRAEDTAVYYCARQTEDRSYGYDLDYWGQGTLVTVSS

SEQ ID NO: 129 - protein, 122 aa, synthetic construct
EVQLVESGGGLVQPGGSLRLSCAASGYSFYSYAMSWVRQAPGKGLEWVSRISQGGGVTHYADSVKGRFTISRDNSKNTLYLQMNSLRAEDTAVYYCARQTEDRSYGYDLDYWGQGTLVTVSS

SEQ ID NO: 130 - protein, 122 aa, synthetic construct
EVQLVESGGGLVQPGGSLRLSCAASGYNFTNSAMSWVRQAPGKGLEWVSSIYYHSGVPRYADSVKGRFTISRDNSKNTLYLQMNSLRAEDTAVYYCARQTEDRSYGYDLDYWGQGTLVTVSS

SEQ ID NO: 131 - protein, 122 aa, synthetic construct
EVQLVESGGGLVQPGGSLRLSCAASGFNFDNYAMSWVRQAPGKGLEWVSRIYGWDWYASYADSVKGRFTISRDNSKNTLYLQMNSLRAEDTAVYYCARQTEDRSYGYDLDYWGQGTLVTVSS

SEQ ID NO: 132 - protein, 122 aa, synthetic construct
EVQLVESGGGLVQPGGSLRLSCAASGYSFGGYAMSWVRQAPGKGLEWVSRISGIKAYNDYADSVKGRFTISRDNSKNTLYLQMNSLRAEDTAVYYCARQTEDRSYGYDLDYWGQGTLVTVSS

SEQ ID NO: 133 - protein, 122 aa, synthetic construct
EVQLVESGGGLVQPGGSLRLSCAASGDSFTGYAMSWVRQAPGKGLEWVSAISGSGGSTYYADSVKGRFTISRDNSKNTLYLQMNSLRAEDTAVYYCARQTEDRSYGYDLDYWGQGTLVTVSS

SEQ ID NO: 134 - protein, 122 aa, synthetic construct
EVQLVESGGGLVQPGGSLRLSCAASGDIFGSYAMSWVRQAPGKGLEWVSAISGSGGSTYYADSVKGRFTISRDNSKNTLYLQMNSLRAEDTAVYYCARQTEDRSYGYDLDYWGQGTLVTVSS

SEQ ID NO: 135 - protein, 122 aa, synthetic construct
EVQLVESGGGLVQPGGSLRLSCAASGFNFGNYAMSWVRQAPGKGLEWVSAIYSYFDEPRYADSVKGRFTISRDNSKNTLYLQMNSLRAEDTAVYYCARQTEDRSYGYDLDYWGQGTLVTVSS

SEQ ID NO: 136 - protein, 126 aa, synthetic construct
EVQLVESGGGLVQPGGSLRLSCAASGFSFDNYDMSWVRQAPGKGLEWVSSIKPGSAYKFYADSVKGRFTISRDNSKNTLYLQMNSLRAEDTAVYYCAREYSDVVDYVSVRTPLDYWGQGTLVTVSS

SEQ ID NO: 137 - protein, 126 aa, synthetic construct
EVQLVESGGGLVQPGGSLRLSCAASGYSFSNYDMSWVRQAPGKGLEWVSGIKGWKSYTGYADSVKGRFTISRDNSKNTLYLQMNSLRAEDTAVYYCAREYSDVVDYVSVRTPLDYWGQGTLVTVSS

SEQ ID NO: 138 - protein, 126 aa, synthetic construct
EVQLVESGGGLVQPGGSLRLSCAASGFSFGNYWMSWVRQAPGKGLEWVSGIDGHSSYAFYADSVKGRFTISRDNSKNTLYLQMNSLRAEDTAVYYCAREYSDVVDYVSVRTPLDYWGQGTLVTVSS

SEQ ID NO: 139 - protein, 126 aa, synthetic construct
EVQLVESGGGLVQPGGSLRLSCAASGFNFTDYWMSWVRQAPGKGLEWVSSIIGDDSTNHYADSVKGRFTISRDNSKNTLYLQMNSLRAEDTAVYYCAREYSDVVDYVSVRTPLDYWGQGTLVTVSS

SEQ ID NO: 140 - protein, 126 aa, synthetic construct
EVQLVESGGGLVQPGGSLRLSCAASGFNFSGFDMSWVRQAPGKGLEWVSGIKAYKSTADYADSVKGRFTISRDNSKNTLYLQMNSLRAEDTAVYYCAREYSDVVDYVSVRTPLDYWGQGTLVTVSS

SEQ ID NO: 141 - protein, 126 aa, synthetic construct
EVQLVESGGGLVQPGGSLRLSCAASGFNFDNYYMSWVRQAPGKGLEWVSSIYQTDASIFYADSVKGRFTISRDNSKNTLYLQMNSLRAEDTAVYYCAREYSDVVDYVSVRTPLDYWGQGTLVTVSS

SEQ ID NO: 142 - protein, 126 aa, synthetic construct
EVQLVESGGGLVQPGGSLRLSCAASGYSFSDYWMSWVRQAPGKGLEWVSSIKQTGGVKHYADSVKGRFTISRDNSKNTLYLQMNSLRAEDTAVYYCAREYSDVVDYVSVRTPLDYWGQGTLVTVSS

SEQ ID NO: 143 - protein, 126 aa, synthetic construct; identical to SEQ ID NO: 139

SEQ ID NO: 144 - protein, 126 aa, synthetic construct
EVQLVESGGGLVQPGGSLRLSCAASGDSFDNYWMSWVRQAPGKGLEWVSAIDTHSDNSFYADSVKGRFTISRDNSKNTLYLQMNSLRAEDTAVYYCAREYSDVVDYVSVRTPLDYWGQGTLVTVSS

SEQ ID NO: 145 - protein, 126 aa, synthetic construct
EVQLVESGGGLVQPGGSLRLSCAASGYNFGSYDMSWVRQAPGKGLEWVSGIKTYGGNTHYADSVKGRFTISRDNSKNTLYLQMNSLRAEDTAVYYCAREYSDVVDYVSVRTPLDYWGQGTLVTVSS

SEQ ID NO: 146 - protein, 126 aa, synthetic construct
EVQLVESGGGLVQPGGSLRLSCAASGFSFYDYDMSWVRQAPGKGLEWVSSIIQSGSTAFYADSVKGRFTISRDNSKNTLYLQMNSLRAEDTAVYYCAREYSDVVDYVSVRTPLDYWGQGTLVTVSS

SEQ ID NO: 147 - protein, 126 aa, synthetic construct
EVQLVESGGGLVQPGGSLRLSCAASGFIFSDFDMSWVRQAPGKGLEWVSGIKQSSAGINYADSVKGRFTISRDNSKNTLYLQMNSLRAEDTAVYYCAREYSDVVDYVSVRTPLDYWGQGTLVTVSS

SEQ ID NO: 148 - protein, 126 aa, synthetic construct
EVQLVESGGGLVQPGGSLRLSCAASGDIFGNYWMSWVRQAPGKGLEWVSSIDASSGNRFYADSVKGRFTISRDNSKNTLYLQMNSLRAEDTAVYYCAREYSDVVDYVSVRTPLDYWGQGTLVTVSS

SEQ ID NO: 149 - protein, 126 aa, synthetic construct
EVQLVESGGGLVQPGGSLRLSCAASGDTFDTYAMSWVRQAPGKGLEWVSGISQWGAYASYADSVKGRFTISRDNSKNTLYLQMNSLRAEDTAVYYCAREYSDVVDYVSVRTPLDYWGQGTLVTVSS

SEQ ID NO: 150 - protein, 126 aa, synthetic construct
EVQLVESGGGLVQPGGSLRLSCAASGYNFSSYDMSWVRQAPGKGLEWVSGISDTGDYANYADSVKGRFTISRDNSKNTLYLQMNSLRAEDTAVYYCAREYSDVVDYVSVRTPLDYWGQGTLVTVSS

SEQ ID NO: 151 - protein, 126 aa, synthetic construct
EVQLVESGGGLVQPGGSLRLSCAASGFSFSNYWMSWVRQAPGKGLEWVSAISPGDGTIFYADSVKGRFTISRDNSKNTLYLQMNSLRAEDTAVYYCAREYSDVVDYVSVRTPLDYWGQGTLVTVSS

SEQ ID NO: 152 - protein, 126 aa, synthetic construct
EVQLVESGGGLVQPGGSLRLSCAASGYNFTNYYMSWVRQAPGKGLEWVSSISAYSDNRNYADSVKGRFTISRDNSKNTLYLQMNSLRAEDTAVYYCAREYSDVVDYVSVRTPLDYWGQGTLVTVSS

SEQ ID NO: 153 - protein, 126 aa, synthetic construct
EVQLVESGGGLVQPGGSLRLSCAASGYTFTDYDMSWVRQAPGKGLEWVSSIITDGGGAFYADSVKGRFTISRDNSKNTLYLQMNSLRAEDTAVYYCAREYSDVVDYVSVRTPLDYWGQGTLVTVSS

SEQ ID NO: 154 - protein, 126 aa, synthetic construct
EVQLVESGGGLVQPGGSLRLSCAASGFSFGGFDMSWVRQAPGKGLEWVSGIKTYGGYRSYADSVKGRFTISRDNSKNTLYLQMNSLRAEDTAVYYCAREYSDVVDYVSVRTPLDYWGQGTLVTVSS

SEQ ID NO: 155 - protein, 126 aa, synthetic construct
EVQLVESGGGLVQPGGSLRLSCAASGYTFDSSWMSWVRQAPGKGLEWVSSIDAYGDYNFYADSVKGRFTISRDNSKNTLYLQMNSLRAEDTAVYYCAREYSDVVDYVSVRTPLDYWGQGTLVTVSS

SEQ ID NO: 156 - protein, 126 aa, synthetic construct
EVQLVESGGGLVQPGGSLRLSCAASGYNFGDYDMSWVRQAPGKGLEWVSSIIGHGDTKFYADSVKGRFTISRDNSKNTLYLQMNSLRAEDTAVYYCAREYSDVVDYVSVRTPLDYWGQGTLVTVSS

SEQ ID NO: 157 - protein, 126 aa, synthetic construct
EVQLVESGGGLVQPGGSLRLSCAASGFNFSDFDMSWVRQAPGKGLEWVSVIKPSGDYINYADSVKGRFTISRDNSKNTLYLQMNSLRAEDTAVYYCAREYSDVVDYVSVRTPLDYWGQGTLVTVSS

SEQ ID NO: 158 - protein, 126 aa, synthetic construct
EVQLVESGGGLVQPGGSLRLSCAASGYSFGNFDMSWVRQAPGKGLEWVSGIKQYKGYTSYADSVKGRFTISRDNSKNTLYLQMNSLRAEDTAVYYCAREYSDVVDYVSVRTPLDYWGQGTLVTVSS

SEQ ID NO: 159 - protein, 126 aa, synthetic construct
EVQLVESGGGLVQPGGSLRLSCAASGFNFTNYWMSWVRQAPGKGLEWVSAISGTGGYTYYADSVKGRFTISRDNSKNTLYLQMNSLRAEDTAVYYCAREYSDVVDYVSVRTPLDYWGQGTLVTVSS

SEQ ID NO: 160 - protein, 126 aa, synthetic construct
EVQLVESGGGLVQPGGSLRLSCAASGFNFYDYDMSWVRQAPGKGLEWVSGIKTHSGGNGYADSVKGRFTISRDNSKNTLYLQMNSLRAEDTAVYYCAREYSDVVDYVSVRTPLDYWGQGTLVTVSS

SEQ ID NO: 161 - protein, 126 aa, synthetic construct
EVQLVESGGGLVQPGGSLRLSCAASGYSFDTYDMSWVRQAPGKGLEWVSGIKQYKGYTSYADSVKGRFTISRDNSKNTLYLQMNSLRAEDTAVYYCAREYSDVVDYVSVRTPLDYWGQGTLVTVSS

SEQ ID NO: 162 - protein, 126 aa, synthetic construct
EVQLVESGGGLVQPGGSLRLSCAASGYTFTGFWMSWVRQAPGKGLEWVSSISPDSGTKHYADSVKGRFTISRDNSKNTLYLQMNSLRAEDTAVYYCAREYSDVVDYVSVRTPLDYWGQGTLVTVSS

SEQ ID NO: 163 - protein, 126 aa, synthetic construct
EVQLVESGGGLVQPGGSLRLSCAASGYTFDDYDMSWVRQAPGKGLEWVSGIKAHSDNKRYADSVKGRFTISRDNSKNTLYLQMNSLRAEDTAVYYCAREYSDVVDYVSVRTPLDYWGQGTLVTVSS

SEQ ID NO: 164 - protein, 126 aa, synthetic construct
EVQLVESGGGLVQPGGSLRLSCAASGYSFTDYDMSWVRQAPGKGLEWVSGIKTYKSDARYADSVKGRFTISRDNSKNTLYLQMNSLRAEDTAVYYCAREYSDVVDYVSVRTPLDYWGQGTLVTVSS

SEQ ID NO: 165 - protein, 126 aa, synthetic construct
EVQLVESGGGLVQPGGSLRLSCAASGYTFTDYDMSWVRQAPGKGLEWVSGIKQYKGYTSYADSVKGRFTISRDNSKNTLYLQMNSLRAEDTAVYYCAREYSDVVDYVSVRTPLDYWGQGTLVTVSS

SEQ ID NO: 166 - protein, 126 aa, synthetic construct
EVQLVESGGGLVQPGGSLRLSCAASGGSFTNYWMSWVRQAPGKGLEWVSVIDSTGSNRFYADSVKGRFTISRDNSKNTLYLQMNSLRAEDTAVYYCAREYSDVVDYVSVRTPLDYWGQGTLVTVSS

SEQ ID NO: 167 - protein, 126 aa, synthetic construct
EVQLVESGGGLVQPGGSLRLSCAASGFNFSNYWMSWVRQAPGKGLEWVSVIDAHSANIRYADSVKGRFTISRDNSKNTLYLQMNSLRAEDTAVYYCAREYSDVVDYVSVRTPLDYWGQGTLVTVSS

SEQ ID NO: 168 - protein, 126 aa, synthetic construct
EVQLVESGGGLVQPGGSLRLSCAASGYSFGDYWMSWVRQAPGKGLEWVSVIDSGSGNKRYADSVKGRFTISRDNSKNTLYLQMNSLRAEDTAVYYCAREYSDVVDYVSVRTPLDYWGQGTLVTVSS

SEQ ID NO: 169 - protein, 126 aa, synthetic construct
EVQLVESGGGLVQPGGSLRLSCAASGFNFGGFDMSWVRQAPGKGLEWVSGIKQYKGYTSYADSVKGRFTISRDNSKNTLYLQMNSLRAEDTAVYYCAREYSDVVDYVSVRTPLDYWGQGTLVTVSS

SEQ ID NO: 170 - protein, 126 aa, synthetic construct
EVQLVESGGGLVQPGGSLRLSCAASGYNFGDYSMSWVRQAPGKGLEWVSVIDTTSAYTRYADSVKGRFTISRDNSKNTLYLQMNSLRAEDTAVYYCAREYSDVVDYVSVRTPLDYWGQGTLVTVSS

SEQ ID NO: 171 - protein, 126 aa, synthetic construct
EVQLVESGGGLVQPGGSLRLSCAASGFTFTTYDMSWVRQAPGKGLEWVSGIKYSKYYTHYADSVKGRFTISRDNSKNTLYLQMNSLRAEDTAVYYCAREYSDVVDYVSVRTPLDYWGQGTLVTVSS

SEQ ID NO: 172 - protein, 126 aa, synthetic construct
EVQLVESGGGLVQPGGSLRLSCAASGYTFDSYWMSWVRQAPGKGLEWVSAIDGTDSVAYYADSVKGRFTISRDNSKNTLYLQMNSLRAEDTAVYYCAREYSDVVDYVSVRTPLDYWGQGTLVTVSS

SEQ ID NO: 173 - protein, 126 aa, synthetic construct
EVQLVESGGGLVQPGGSLRLSCAASGFSFGDYWMSWVRQAPGKGLEWVSAIDQGKATSFYADSVKGRFTISRDNSKNTLYLQMNSLRAEDTAVYYCAREYSDVVDYVSVRTPLDYWGQGTLVTVSS

SEQ ID NO: 174 - protein, 126 aa, synthetic construct
EVQLVESGGGLVQPGGSLRLSCAASGFNFGNYDMSWVRQAPGKGLEWVSSIIPHGDYSFYADSVKGRFTISRDNSKNTLYLQMNSLRAEDTAVYYCAREYSDVVDYVSVRTPLDYWGQGTLVTVSS

SEQ ID NO: 175 - protein, 126 aa, synthetic construct
EVQLVESGGGLVQPGGSLRLSCAASGYNFTSYDMSWVRQAPGKGLEWVSGIKTGGGSARYADSVKGRFTISRDNSKNTLYLQMNSLRAEDTAVYYCAREYSDVVDYVSVRTPLDYWGQGTLVTVSS

SEQ ID NO: 176 - protein, 126 aa, synthetic construct
EVQLVESGGGLVQPGGSLRLSCAASGYNFTDYDMSWVRQAPGKGLEWVSSIIASGSGNYYADSVKGRFTISRDNSKNTLYLQMNSLRAEDTAVYYCAREYSDVVDYVSVRTPLDYWGQGTLVTVSS

SEQ ID NO: 177 - protein, 126 aa, synthetic construct
EVQLVESGGGLVQPGGSLRLSCAASGYIFTNYWMSWVRQAPGKGLEWVSSIDQGSGNIFYADSVKGRFTISRDNSKNTLYLQMNSLRAEDTAVYYCAREYSDVVDYVSVRTPLDYWGQGTLVTVSS

SEQ ID NO: 178 - protein, 126 aa, synthetic construct
EVQLVESGGGLVQPGGSLRLSCAASGDSFTNYWMSWVRQAPGKGLEWVSGISQGGSYAYYADSVKGRFTISRDNSKNTLYLQMNSLRAEDTAVYYCAREYSDVVDYVSVRTPLDYWGQGTLVTVSS

SEQ ID NO: 179 - protein, 126 aa, synthetic construct
EVQLVESGGGLVQPGGSLRLSCAASGFSFGDFAMSWVRQAPGKGLEWVSVIDGHTAYNSYADSVKGRFTISRDNSKNTLYLQMNSLRAEDTAVYYCAREYSDVVDYVSVRTPLDYWGQGTLVTVSS

SEQ ID NO: 180 - protein, 126 aa, synthetic construct
EVQLVESGGGLVQPGGSLRLSCAASGFIFDGYDMSWVRQAPGKGLEWVSVIKDHGGYKFYADSVKGRFTISRDNSKNTLYLQMNSLRAEDTAVYYCAREYSDVVDYVSVRTPLDYWGQGTLVTVSS

SEQ ID NO: 181 - protein, 5 aa, synthetic construct
NYAMS

SEQ ID NO: 182 - protein, 5 aa, synthetic construct
TYGMS

SEQ ID NO: 183 - protein, 5 aa, synthetic construct
SYGMS

SEQ ID NO: 184 - protein, 5 aa, synthetic construct
DYGMS

SEQ ID NO: 185 - protein, 5 aa, synthetic construct
NYSMS

SEQ ID NO: 186 - protein, 5 aa, synthetic construct
GFGMS

SEQ ID NO: 187 - protein, 5 aa, synthetic construct
DYAMS

SEQ ID NO: 188 - protein, 5 aa, synthetic construct
GSSMS

SEQ ID NO: 189 - protein, 5 aa, synthetic construct
NYGMS

SEQ ID NO: 190 - protein, 5 aa, synthetic construct
GYGMS

SEQ ID NO: 191 - protein, 5 aa, synthetic construct
TFYMS

SEQ ID NO: 192 - protein, 5 aa, synthetic construct
DFGMS

SEQ ID NO: 193 - protein, 5 aa, synthetic construct
NSGMS

SEQ ID NO: 194 - protein, 5 aa, synthetic construct
GYSMS

SEQ ID NO: 195 - protein, 5 aa, synthetic construct
SSGMS

SEQ ID NO: 196 - protein, 17 aa, synthetic construct
RISPTGGYASYADSVKG

SEQ ID NO: 197 - protein, 17 aa, synthetic construct
GIKPGDSTTYYADSVKG

SEQ ID NO: 198 - protein, 17 aa, synthetic construct
GIKWITGESYYADSVKG

SEQ ID NO: 199 - protein, 17 aa, synthetic construct
GIKPWGSGTYYADSVKG

SEQ ID NO: 200 - protein, 17 aa, synthetic construct
GIYPSGDNNRYADSVKG

SEQ ID NO: 201 - protein, 17 aa, synthetic construct
GISGSGDNKYYADSVKG

SEQ ID NO: 202 - protein, 17 aa, synthetic construct
GIYSHDADKRYADSVKG

SEQ ID NO: 203 - protein, 17 aa, synthetic construct
IIYPTGSTNYYADSVKG

SEQ ID NO: 204 - protein, 17 aa, synthetic construct
RISPYTDNKYYADSVKG

SEQ ID NO: 205 - protein, 17 aa, synthetic construct
RISGDSANIRYADSVKG

SEQ ID NO: 206 - protein, 17 aa, synthetic construct
GIKPSSWTTYYADSVKG

SEQ ID NO: 207 - protein, 17 aa, synthetic construct
GIYASGSDKRYADSVKG

SEQ ID NO: 208 - protein, 17 aa, synthetic construct
RISGDGSNINYADSVKG

SEQ ID NO: 209 - protein, 17 aa, synthetic construct
GISPSGGTIGYADSVKG

SEQ ID NO: 210 - protein, 17 aa, synthetic construct
RIDPWGASIRYADSVKG

SEQ ID NO: 211 - protein, 17 aa, synthetic construct
GIKPSTSTTYYADSVKG

SEQ ID NO: 212 - protein, 17 aa, synthetic construct
GIYPSGDSRRYADSVKG

SEQ ID NO: 213 - protein, 17 aa, synthetic construct
RISQWGDTSNYADSVKG

SEQ ID NO: 214 - protein, 17 aa, synthetic construct
GIKPHSDVAHYADSVKG

SEQ ID NO: 215 - protein, 17 aa, synthetic construct
GIKPTGSYINYADSVKG

SEQ ID NO: 216 - protein, 17 aa, synthetic construct
GIKPTGASTYYADSVKG

SEQ ID NO: 217 - protein, 17 aa, synthetic construct
GIKPDSATTYYADSVKG

SEQ ID NO: 218 - protein, 17 aa, synthetic construct
IISPDGGYKRYADSVKG

SEQ ID NO: 219 - protein, 17 aa, synthetic construct
RIDPSGWSTSYADSVKG

SEQ ID NO: 220 - protein, 17 aa, synthetic construct
GIKPHTDDIYYADSVKG

SEQ ID NO: 221 - protein, 17 aa, synthetic construct
RIKSDGGDTHYADSVKG

SEQ ID NO: 222 - protein, 17 aa, synthetic construct
RISPGDSTPRYADSVKG

SEQ ID NO: 223 - protein, 17 aa, synthetic construct
RISPYTGTTHYADSVKG

SEQ ID NO: 224 - protein, 17 aa, synthetic construct
RISPSKAVKDYADSVKG

SEQ ID NO: 225 - protein, 17 aa, synthetic construct
GIKWSSDETYYADSVKG

SEQ ID NO: 226 - protein, 17 aa, synthetic construct
WISPSKGSASYADSVKG

SEQ ID NO: 227 - protein, 17 aa, synthetic construct
GIYQTGSNTRYADSVKG

SEQ ID NO: 228 - protein, 17 aa, synthetic construct
RIDWDGGNTRYADSVKG

SEQ ID NO: 229 - protein, 17 aa, synthetic construct
RISQYGGGIRYADSVKG

SEQ ID NO: 230 - protein, 17 aa, synthetic construct
RIKPTDGSTHYADSVKG

SEQ ID NO: 231 - protein, 17 aa, synthetic construct
WISAWDGSIYYADSVKG

SEQ ID NO: 232 - protein, 453 aa, synthetic construct
EVQLVESGGGLVQPGGSLRLSCAASGFTFSSYAMSWVRQAPGKGLEWVSAISGSGGSTYYADSVKGRFTISRDNSKNTLYLQMNSLRAEDTAVYYCARAELLAFDVYTASDYWGQGTLVTVSSASTKGPSVFPLAPSSKSTSGGTAALGCLVKDYFPEPVTVSWNSGALTSGVHTFPAVLQSSGLYSLSSVVTVPSSSLGTQTYICNVNHKPSNTKVDKKVEPKSCDKTHTCPPCPAPELLGGPSVFLFPPKPKDTLMISRTPEVTCVVVDVSHEDPEVKFNWYVDGVEVHNAKTKPREEQYNSTYRVVSVLTVLHQDWLNGKEYKCKVSNKALPAPIEKTISKAKGQPREPQVYTLPPSRDELTKNQVSLTCLVKGFYPSDIAVEWESNGQPENNYKTTPPVLDSDGSFFLYSKLTVDKSRWQQGNVFSCSVMHEALHNHYTQKSLSLSPGK

SEQ ID NO: 233 - protein, 452 aa, synthetic construct
EVQLVESGGGLVQPGGSLRLSCAASGFTFSSYAMSWVRQAPGKGLEWVSAISGSGGSTYYADSVKGRFTISRDNSKNTLYLQMNSLRAEDTAVYYCARQTEDRSYGYDLDYWGQGTLVTVSSASTKGPSVFPLAPSSKSTSGGTAALGCLVKDYFPEPVTVSWNSGALTSGVHTFPAVLQSSGLYSLSSVVTVPSSSLGTQTYICNVNHKPSNTKVDKKVEPKSCDKTHTCPPCPAPELLGGPSVFLFPPKPKDTLMISRTPEVTCVVVDVSHEDPEVKFNWYVDGVEVHNAKTKPREEQYNSTYRVVSVLTVLHQDWLNGKEYKCKVSNKALPAPIEKTISKAKGQPREPQVYTLPPSRDELTKNQVSLTCLVKGFYPSDIAVEWESNGQPENNYKTTPPVLDSDGSFFLYSKLTVDKSRWQQGNVFSCSVMHEALHNHYTQKSLSLSPGK

SEQ ID NO: 234 - protein, 5 aa, synthetic construct
TNAMS

SEQ ID NO: 235 - protein, 5 aa, synthetic construct
DYSMS

SEQ ID NO: 236 - protein, 5 aa, synthetic construct
SSAMS

SEQ ID NO: 237 - protein, 5 aa, synthetic construct
GYAMS

SEQ ID NO: 238 - protein, 5 aa, synthetic construct
TYAMS

SEQ ID NO: 239 - protein, 4 aa, synthetic construct
TYMS

SEQ ID NO: 240 - protein, 5 aa, synthetic construct
TSAMS

SEQ ID NO: 241 - protein, 5 aa, synthetic construct
DFAMS

SEQ ID NO: 242 - protein, 5 aa, synthetic construct
GFAMS

SEQ ID NO: 243 - protein, 5 aa, synthetic construct
SNAMS

SEQ ID NO: 244 - protein, 5 aa, synthetic construct
NNAMS

SEQ ID NO: 245 - protein, 5 aa, synthetic construct
TSSMS

SEQ ID NO: 246 - protein, 5 aa, synthetic construct
NFAMS

SEQ ID NO: 247 - protein, 5 aa, synthetic construct
GNAMS

SEQ ID NO: 248 - protein, 5 aa, synthetic construct
NSAMS

SEQ ID NO: 249 - protein, 456 aa, synthetic construct
EVQLVESGGGLVQPGGSLRLSCAASGFTFSSYAMSWVRQAPGKGLEWVSAISGSGGSTYYADSVKGRFTISRDNSKNTLYLQMNSLRAEDTAVYYCAREYSDVVDYVSVRTPLDYWGQGTLVTVSSASTKGPSVFPLAPSSKSTSGGTAALGCLVKDYFPEPVTVSWNSGALTSGVHTFPAVLQSSGLYSLSSVVTVPSSSLGTQTYICNVNHKPSNTKVDKKVEPKSCDKTHTCPPCPAPELLGGPSVFLFPPKPKDTLMISRTPEVTCVVVDVSHEDPEVKFNWYVDGVEVHNAKTKPREEQYNSTYRVVSVLTVLHQDWLNGKEYKCKVSNKALPAPIEKTISKAKGQPREPQVYTLPPSRDELTKNQVSLTCLVKGFYPSDIAVEWESNGQPENNYKTTPPVLDSDGSFFLYSKLTVDKSRWQQGNVFSCSVMHEALHNHYTQKSLSLSPGK

SEQ ID NO: 250 - protein, 214 aa, synthetic construct
DIQMTQSPSSLSASVGDRVTITCRASQGISSYLAWYQQKPGKAPKLLIYAASSLQSGVPSRFSGSGSGTDFTLTISSLQPEDFATYYCQQHYTTPPTFGQGTKVEIKRTVAAPSVFIFPPSDEQLKSGTASVVCLLNNFYPREAKVQWKVDNALQSGNSQESVTEQDSKDSTYSLSSTLTLSKADYEKHKVYACEVTHQGLSSPVTKSFNRGEC

SEQ ID NO: 251 - protein, 17 aa, synthetic construct
AISTGGDNKRYADSVKG

SEQ ID NO: 252 - protein, 17 aa, synthetic construct
RIYPGSWSPDYADSVKG

SEQ ID NO: 253 - protein, 17 aa, synthetic construct
RIKTTDDGKSYADSVKG

SEQ ID NO: 254 - protein, 17 aa, synthetic construct
AIDASGGDTRYADSVKG

SEQ ID NO: 255 - protein, 17 aa, synthetic construct
RISAWGSTNNYADSVKG

SEQ ID NO: 256 - protein, 17 aa, synthetic construct
RISTGFAGPDYADSVKG

SEQ ID NO: 257 - protein, 17 aa, synthetic construct
RIKASSGGSDYADSVKG

SEQ ID NO: 258 - protein, 17 aa, synthetic construct
AISGSSDSPRYADSVKG

SEQ ID NO: 259 - protein, 17 aa, synthetic construct
RIDGTGDSKFYADSVKG

SEQ ID NO: 260 - protein, 17 aa, synthetic construct
WIDTTSAYASYADSVKG

SEQ ID NO: 261 - protein, 17 aa, synthetic construct
RISGSGDGKDYADSVKG

SEQ ID NO: 262 - protein, 17 aa, synthetic construct
RISAHKWDASYADSVKG

SEQ ID NO: 263 - protein, 17 aa, synthetic construct
RIYTDGWEKDYADSVKG

SEQ ID NO: 264 - protein, 17 aa, synthetic construct
RISSYSWNPDYADSVKG

SEQ ID NO: 265 - protein, 17 aa, synthetic construct
RISQTGGTTDYADSVKG

SEQ ID NO: 266 - protein, 16 aa, synthetic construct
RIYTDGSSDYADSVKG

SEQ ID NO: 267 - protein, 17 aa, synthetic construct
AIDAIGGNKRYADSVKG

SEQ ID NO: 268 - protein, 17 aa, synthetic construct
RIYSISGNTDYADSVKG

SEQ ID NO: 269 - protein, 17 aa, synthetic construct
RISGISAGTNYADSVKG

SEQ ID NO: 270 - protein, 17 aa, synthetic construct
RIYADTAYNDYADSVKG

SEQ ID NO: 271 - protein, 17 aa, synthetic construct
RIYSGDDNASYADSVKG

SEQ ID NO: 272 - protein, 17 aa, synthetic construct
RIYPYSSVRDYADSVKG

SEQ ID NO: 273 - protein, 17 aa, synthetic construct
RIYPTSSESDYADSVKG

SEQ ID NO: 274 - protein, 17 aa, synthetic construct
RISGHDWSSSYADSVKG

SEQ ID NO: 275 - protein, 17 aa, synthetic construct
RISSDGWETFYADSVKG

SEQ ID NO: 276 - protein, 17 aa, synthetic construct
RIYGGSWDTDYADSVKG

SEQ ID NO: 277 - protein, 17 aa, synthetic construct
RISAYGWGKSYADSVKG

SEQ ID NO: 278 - protein, 17 aa, synthetic construct
RIDTIGGTSSYADSVKG

SEQ ID NO: 279 - protein, 17 aa, synthetic construct
RIDTWGWYKFYADSVKG

SEQ ID NO: 280 - protein, 17 aa, synthetic construct
RIYQDSSTTDYADSVKG

SEQ ID NO: 281 - protein, 17 aa, synthetic construct
RIKSHDSTSHYADSVKG

SEQ ID NO: 282 - protein, 17 aa, synthetic construct
RIYAYKSENDYADSVKG

SEQ ID NO: 283 - protein, 17 aa, synthetic construct
RIYGSDSTPDYADSVKG

SEQ ID NO: 284 - protein, 17 aa, synthetic construct
RISQDGGNKNYADSVKG

SEQ ID NO: 285 - protein, 17 aa, synthetic construct
RIDGWGSYTDYADSVKG

SEQ ID NO: 286 - protein, 17 aa, synthetic construct
RISGTSGNNDYADSVKG

SEQ ID NO: 287 - protein, 17 aa, synthetic construct
RISAHSWNKDYADSVKG

SEQ ID NO: 288 - protein, 17 aa, synthetic construct
RISADSASPSYADSVKG

SEQ ID NO: 289 - protein, 17 aa, synthetic construct
RIDTGGSVKNYADSVKG

SEQ ID NO: 290 - protein, 17 aa, synthetic construct
RISPSTWNIDYADSVKG

SEQ ID NO: 291 - protein, 17 aa, synthetic construct
RISPDSSGISYADSVKG

SEQ ID NO: 292 - protein, 17 aa, synthetic construct
RISSHGASRDYADSVKG

SEQ ID NO: 293 - protein, 17 aa, synthetic construct
AIYASTDGRSYADSVKG

SEQ ID NO: 294 - protein, 17 aa, synthetic construct
RISSDKGTTNYADSVKG

SEQ ID NO: 295 - protein, 17 aa, synthetic construct
RISTDGAYTNYADSVKG

SEQ ID NO: 296 - protein, 17 aa, synthetic construct
RIYSTKGTPDYADSVKG

SEQ ID NO: 297 - protein, 17 aa, synthetic construct
RISTYGDTTHYADSVKG

SEQ ID NO: 298 - protein, 17 aa, synthetic construct
RISQSGGTNDYADSVKG

SEQ ID NO: 299 - protein, 17 aa, synthetic construct
RISQGGGVTHYADSVKG

SEQ ID NO: 300 - protein, 17 aa, synthetic construct
SIYYHSGVPRYADSVKG

SEQ ID NO: 301 - protein, 17 aa, synthetic construct
RIYGWDWYASYADSVKG

SEQ ID NO: 302 - protein, 17 aa, synthetic construct
RISGIKAYNDYADSVKG

SEQ ID NO: 303 - protein, 17 aa, synthetic construct
AIYSYFDEPRYADSVKG

SEQ ID NO: 304 - protein, 5 aa, synthetic construct
NYDMS

SEQ ID NO: 305 - protein, 5 aa, synthetic construct
NYWMS

SEQ ID NO: 306 - protein, 5 aa, synthetic construct
DYWMS

SEQ ID NO: 307 - protein, 5 aa, synthetic construct
GFDMS

SEQ ID NO: 308 - protein, 5 aa, synthetic construct
NYYMS

SEQ ID NO: 309 - protein, 5 aa, synthetic construct
SYDMS

SEQ ID NO: 310 - protein, 5 aa, synthetic construct
DYDMS

SEQ ID NO: 311 - protein, 5 aa, synthetic construct
DFDMS

SEQ ID NO: 312 - protein, 5 aa, synthetic construct
SSWMS

SEQ ID NO: 313 - protein, 5 aa, synthetic construct
NFDMS

SEQ ID NO: 314 - protein, 5 aa, synthetic construct
TYDMS

SEQ ID NO: 315 - protein, 5 aa, synthetic construct
GFWMS

SEQ ID NO: 316 - protein, 5 aa, synthetic construct
SYWMS

SEQ ID NO: 317 - protein, 5 aa, synthetic construct
GYDMS

SEQ ID NO: 318 - protein, 17 aa, synthetic construct
SIKPGSAYKFYADSVKG

SEQ ID NO: 319 - protein, 17 aa, synthetic construct
GIKGWKSYTGYADSVKG

SEQ ID NO: 320 - protein, 17 aa, synthetic construct
GIDGHSSYAFYADSVKG

SEQ ID NO: 321 - protein, 17 aa, synthetic construct
SIIGDDSTNHYADSVKG

SEQ ID NO: 322 - protein, 17 aa, synthetic construct
GIKAYKSTADYADSVKG

SEQ ID NO: 323 - protein, 17 aa, synthetic construct
SIYQTDASIFYADSVKG

SEQ ID NO: 324 - protein, 17 aa, synthetic construct
SIKQTGGVKHYADSVKG

SEQ ID NO: 325 - protein, 17 aa, synthetic construct
AIDTHSDNSFYADSVKG

SEQ ID NO: 326 - protein, 17 aa, synthetic construct
GIKTYGGNTHYADSVKG

SEQ ID NO: 327 - protein, 17 aa, synthetic construct
SIIQSGSTAFYADSVKG

SEQ ID NO: 328 - protein, 17 aa, synthetic construct
GIKQSSAGINYADSVKG

SEQ ID NO: 329 - protein, 17 aa, synthetic construct
SIDASSGNRFYADSVKG

SEQ ID NO: 330 - protein, 17 aa, synthetic construct
GISQWGAYASYADSVKG

SEQ ID NO: 331 - protein, 17 aa, synthetic construct
GISDTGDYANYADSVKG

SEQ ID NO: 332 - protein, 17 aa, synthetic construct
AISPGDGTIFYADSVKG

SEQ ID NO: 333 - protein, 17 aa, synthetic construct
SISAYSDNRNYADSVKG

SEQ ID NO: 334 - protein, 17 aa, synthetic construct
SIITDGGGAFYADSVKG

SEQ ID NO: 335 - protein, 17 aa, synthetic construct
GIKTYGGYRSYADSVKG

SEQ ID NO: 336 - protein, 17 aa, synthetic construct
SIDAYGDYNFYADSVKG

SEQ ID NO: 337 - protein, 17 aa, synthetic construct
SIIGHGDTKFYADSVKG

SEQ ID NO: 338 - protein, 17 aa, synthetic construct
VIKPSGDYINYADSVKG

SEQ ID NO: 339 - protein, 17 aa, synthetic construct
GIKQYKGYTSYADSVKG

SEQ ID NO: 340 - protein, 17 aa, synthetic construct
AISGTGGYTYYADSVKG

SEQ ID NO: 341 - protein, 17 aa, synthetic construct
GIKTHSGGNGYADSVKG

SEQ ID NO: 342 - protein, 17 aa, synthetic construct
SISPDSGTKHYADSVKG

SEQ ID NO: 343 - protein, 17 aa, synthetic construct
GIKAHSDNKRYADSVKG

SEQ ID NO: 344 - protein, 17 aa, synthetic construct
GIKTYKSDARYADSVKG

SEQ ID NO: 345 - protein, 17 aa, synthetic construct
VIDSTGSNRFYADSVKG

SEQ ID NO: 346 - protein, 17 aa, synthetic construct
VIDAHSANIRYADSVKG

SEQ ID NO: 347 - protein, 17 aa, synthetic construct
VIDSGSGNKRYADSVKG

SEQ ID NO: 348 - protein, 17 aa, synthetic construct
VIDTTSAYTRYADSVKG

SEQ ID NO: 349 - protein, 17 aa, synthetic construct
GIKYSKYYTHYADSVKG

SEQ ID NO: 350 - protein, 17 aa, synthetic construct
AIDGTDSVAYYADSVKG

SEQ ID NO: 351 - protein, 17 aa, synthetic construct
AIDQGKATSFYADSVKG

SEQ ID NO: 352 - protein, 17 aa, synthetic construct
SIIPHGDYSFYADSVKG

SEQ ID NO: 353 - protein, 17 aa, synthetic construct
GIKTGGGSARYADSVKG

SEQ ID NO: 354 - protein, 17 aa, synthetic construct
SIIASGSGNYYADSVKG

SEQ ID NO: 355 - protein, 17 aa, synthetic construct
SIDQGSGNIFYADSVKG

SEQ ID NO: 356 - protein, 17 aa, synthetic construct
GISQGGSYAYYADSVKG

SEQ ID NO: 357 - protein, 17 aa, synthetic construct
VIDGHTAYNSYADSVKG

SEQ ID NO: 358 - protein, 17 aa, synthetic construct
VIKDHGGYKFYADSVKG

SEQ ID NO: 359 - DNA, 645 bp, synthetic construct
  source 1..645: mol_type = other DNA
gatatccagatgacccagtcccccagctccctgagcgctagcgtgggcgaccgggtgaccatcacctgcagggcctcccagggcatcagctcctacctggcttggtatcagcagaagcctggcaaggcccctaagctgctgatctatgccgcttcctccctgcagtccggcgtgccttccaggttcagcggctccggcagcggcaccgacttcaccctgaccatctcctccctgcagcctgaggacttcgccacctattattgccagcagcactataccacccctcctacctttggccagggcaccaaggtggagatcaagcgtacggtggctgcaccatctgtcttcatcttcccgccatctgatgagcagttgaaatctggaactgcctctgttgtgtgcctgctgaataacttctatcccagagaggccaaagtacagtggaaggtggataacgccctccaatcgggtaactcccaggagagtgtcacagagcaggacagcaaggacagcacctacagcctcagcagcaccctgacgctgagcaaagcagactacgagaaacacaaagtctacgcctgcgaagtcacccatcagggcctgagctcgcccgtcacaaagagcttcaacaggggagagtgttga

SEQ ID NO: 360 - protein, 456 aa, synthetic construct
EVQLVESGGGLVQPGGSLRLSCAASGFSFGDFAMSWVRQAPGKGLEWVSVIDGHTAYNSYADSVKGRFTISRDNSKNTLYLQMNSLRAEDTAVYYCAREYSDVVDYVSVRTPLDYWGQGTLVTVSSASTKGPSVFPLAPSSKSTSGGTAALGCLVKDYFPEPVTVSWNSGALTSGVHTFPAVLQSSGLYSLSSVVTVPSSSLGTQTYICNVNHKPSNTKVDKKVEPKSCDKTHTCPPCPAPELLGGPSVFLFPPKPKDTLMISRTPEVTCVVVDVSHEDPEVKFNWYVDGVEVHNAKTKPREEQYNSTYRVVSVLTVLHQDWLNGKEYKCKVSNKALPAPIEKTISKAKGQPREPQVYTLPPSRDELTKNQVSLTCLVKGFYPSDIAVEWESNGQPENNYKTTPPVLDSDGSFFLYSKLTVDKSRWQQGNVFSCSVMHEALHNHYTQKSLSLSPGK

SEQ ID NO: 361 - protein, 453 aa, synthetic construct
EVQLVESGGGLVQPGGSLRLSCAASGFSFGTYGMSWVRQAPGKGLEWVSRISGDSANIRYADSVKGRFTISRDNSKNTLYLQMNSLRAEDTAVYYCARAELLAFDVYTASDYWGQGTLVTVSSASTKGPSVFPLAPSSKSTSGGTAALGCLVKDYFPEPVTVSWNSGALTSGVHTFPAVLQSSGLYSLSSVVTVPSSSLGTQTYICNVNHKPSNTKVDKKVEPKSCDKTHTCPPCPAPELLGGPSVFLFPPKPKDTLMISRTPEVTCVVVDVSHEDPEVKFNWYVDGVEVHNAKTKPREEQYNSTYRVVSVLTVLHQDWLNGKEYKCKVSNKALPAPIEKTISKAKGQPREPQVYTLPPSRDELTKNQVSLTCLVKGFYPSDIAVEWESNGQPENNYKTTPPVLDSDGSFFLYSKLTVDKSRWQQGNVFSCSVMHEALHNHYTQKSLSLSPGK

SEQ ID NO: 362 - protein, 453 aa, synthetic construct
EVQLVESGGGLVQPGGSLRLSCAASGFNFDSYAMSWVRQAPGKGLEWVSGIKPHTDDIYYADSVKGRFTISRDNSKNTLYLQMNSLRAEDTAVYYCARAELLAFDVYTASDYWGQGTLVTVSSASTKGPSVFPLAPSSKSTSGGTAALGCLVKDYFPEPVTVSWNSGALTSGVHTFPAVLQSSGLYSLSSVVTVPSSSLGTQTYICNVNHKPSNTKVDKKVEPKSCDKTHTCPPCPAPELLGGPSVFLFPPKPKDTLMISRTPEVTCVVVDVSHEDPEVKFNWYVDGVEVHNAKTKPREEQYNSTYRVVSVLTVLHQDWLNGKEYKCKVSNKALPAPIEKTISKAKGQPREPQVYTLPPSRDELTKNQVSLTCLVKGFYPSDIAVEWESNGQPENNYKTTPPVLDSDGSFFLYSKLTVDKSRWQQGNVFSCSVMHEALHNHYTQKSLSLSPGK

SEQ ID NO: 363 - protein, 452 aa, synthetic construct
EVQLVESGGGLVQPGGSLRLSCAASGFNFSDYSMSWVRQAPGKGLEWVSRIKASSGGSDYADSVKGRFTISRDNSKNTLYLQMNSLRAEDTAVYYCARQTEDRSYGYDLDYWGQGTLVTVSSASTKGPSVFPLAPSSKSTSGGTAALGCLVKDYFPEPVTVSWNSGALTSGVHTFPAVLQSSGLYSLSSVVTVPSSSLGTQTYICNVNHKPSNTKVDKKVEPKSCDKTHTCPPCPAPELLGGPSVFLFPPKPKDTLMISRTPEVTCVVVDVSHEDPEVKFNWYVDGVEVHNAKTKPREEQYNSTYRVVSVLTVLHQDWLNGKEYKCKVSNKALPAPIEKTISKAKGQPREPQVYTLPPSRDELTKNQVSLTCLVKGFYPSDIAVEWESNGQPENNYKTTPPVLDSDGSFFLYSKLTVDKSRWQQGNVFSCSVMHEALHNHYTQKSLSLSPGK

SEQ ID NO: 364 - DNA, 1371 bp, synthetic construct
  source 1..1371: mol_type = other DNA
gaagtgcaattggtggaaagcggcggcggcctggtgcagccgggcggcagcctgcgcctgagctgcgcggcgtccggattctcttttggtgacttcgctatgagctgggtgcgccaggcaccgggcaaaggcctcgaatgggtgagcgttattgacggtcatactgcttacaactcttatgcggatagcgtgaaaggccgctttaccattagccgcgataattcgaaaaacaccctgtatctgcaaatgaacagcctgcgtgcggaagatactgcagtgtattattgcgcgcgtgaatactctgacgttgttgactacgtttctgttcgtactccgctggattattggggccaaggcaccctggtgacggtgagcagcgcctctaccaagggcccctctgtgtttcctctggctccctccagcaagtctacctctggtggaacagctgccctgggctgcctggtcaaggattactttcctgagcctgtcaccgtgtcctggaactctggcgctctgacatctggcgtgcacacctttccagctgtgctccagtcctccggcctgtactctctgtcctctgtcgtgaccgtgccttctagctctctgggcacccagacctacatctgcaatgtgaaccacaagccttccaacaccaaggtggacaagaaggtggaacccaagtcctgcgacaagacccacacctgtcctccatgtcctgctccagaactgctcggcggaccttccgtgttcctgtttcctccaaagcctaaggacaccctgatgatctctcggacccctgaagtgacctgcgtggtggtggatgtgtctcacgaagatcccgaagtgaagttcaactggtacgtggacggcgtggaagtgcacaacgccaagaccaagcctagagaggaacagtacaactccacctacagagtggtgtccgtgctgaccgtgctgcaccaggattggctgaacggcaaagagtacaagtgcaaggtgtccaacaaggccctgcctgctcctatcgaaaagaccatctccaaggccaagggccagcctagggaaccccaggtttacaccttgcctccatctcgggacgagctgaccaagaaccaggtgtccctgacctgtctcgtgaagggcttctacccctccgacatcgccgtggaatgggagtctaatggccagcctgagaacaactacaagacaacccctcctgtgctggactccgacggctcattcttcctgtactccaagctgacagtggacaagtccagatggcagcagggcaacgtgttctcctgctccgtgatgcacgaggccctgcacaatcactacacccagaagtccctgtctctgtcccctggcaaataa

SEQ ID NO: 365 - DNA, 1362 bp, synthetic construct
  source 1..1362: mol_type = other DNA
gaagtgcaattggtggaaagcggcggcggcctggtgcagccgggcggcagcctgcgcctgagctgcgcggcgtccggattctcttttggtacttacggtatgagctgggtgcgccaggcaccgggcaaaggcctcgaatgggtgagccgtatttctggtgactctgctaacatccgttatgcggatagcgtgaaaggccgctttaccattagccgcgataattcgaaaaacaccctgtatctgcaaatgaacagcctgcgtgcggaagatactgcagtgtattattgcgcgcgtgctgaactgctggctttcgacgtttacactgcttctgattattggggccaaggcaccctggtgacggtgagcagcgcctctaccaagggcccctctgtgtttcctctggctccctccagcaagtctacctctggtggaacagctgccctgggctgcctggtcaaggattactttcctgagcctgtcaccgtgtcctggaactctggcgctctgacatctggcgtgcacacctttccagctgtgctccagtcctccggcctgtactctctgtcctctgtcgtgaccgtgccttctagctctctgggcacccagacctacatctgcaatgtgaaccacaagccttccaacaccaaggtggacaagaaggtggaacccaagtcctgcgacaagacccacacctgtcctccatgtcctgctccagaactgctcggcggaccttccgtgttcctgtttcctccaaagcctaaggacaccctgatgatctctcggacccctgaagtgacctgcgtggtggtggatgtgtctcacgaagatcccgaagtgaagttcaactggtacgtggacggcgtggaagtgcacaacgccaagaccaagcctagagaggaacagtacaactccacctacagagtggtgtccgtgctgaccgtgctgcaccaggattggctgaacggcaaagagtacaagtgcaaggtgtccaacaaggccctgcctgctcctatcgaaaagaccatctccaaggccaagggccagcctagggaaccccaggtttacaccttgcctccatctcgggacgagctgaccaagaaccaggtgtccctgacctgtctcgtgaagggcttctacccctccgacatcgccgtggaatgggagtctaatggccagcctgagaacaactacaagacaacccctcctgtgctggactccgacggctcattcttcctgtactccaagctgacagtggacaagtccagatggcagcagggcaacgtgttctcctgctccgtgatgcacgaggccctgcacaatcactacacccagaagtccctgtctctgtcccctggcaaataa

SEQ ID NO: 366 - DNA, 1362 bp, synthetic construct
  source 1..1362: mol_type = other DNA
gaagtgcaattggtggaaagcggcggcggcctggtgcagccgggcggcagcctgcgcctgagctgcgcggcgtccggattcaactttgactcttacgctatgagctgggtgcgccaggcaccgggcaaaggcctcgaatgggtgagcggtattaaaccgcatactgacgacatctactatgcggatagcgtgaaaggccgctttaccattagccgcgataattcgaaaaacaccctgtatctgcaaatgaacagcctgcgtgcggaagatactgcagtgtattattgcgcgcgtgctgaactgctggctttcgacgtttacactgcttctgattattggggccaaggcaccctggtgacggtgagcagcgcctctaccaagggcccctctgtgtttcctctggctccctccagcaagtctacctctggtggaacagctgccctgggctgcctggtcaaggattactttcctgagcctgtcaccgtgtcctggaactctggcgctctgacatctggcgtgcacacctttccagctgtgctccagtcctccggcctgtactctctgtcctctgtcgtgaccgtgccttctagctctctgggcacccagacctacatctgcaatgtgaaccacaagccttccaacaccaaggtggacaagaaggtggaacccaagtcctgcgacaagacccacacctgtcctccatgtcctgctccagaactgctcggcggaccttccgtgttcctgtttcctccaaagcctaaggacaccctgatgatctctcggacccctgaagtgacctgcgtggtggtggatgtgtctcacgaagatcccgaagtgaagttcaactggtacgtggacggcgtggaagtgcacaacgccaagaccaagcctagagaggaacagtacaactccacctacagagtggtgtccgtgctgaccgtgctgcaccaggattggctgaacggcaaagagtacaagtgcaaggtgtccaacaaggccctgcctgctcctatcgaaaagaccatctccaaggccaagggccagcctagggaaccccaggtttacaccttgcctccatctcgggacgagctgaccaagaaccaggtgtccctgacctgtctcgtgaagggcttctacccctccgacatcgccgtggaatgggagtctaatggccagcctgagaacaactacaagacaacccctcctgtgctggactccgacggctcattcttcctgtactccaagctgacagtggacaagtccagatggcagcagggcaacgtgttctcctgctccgtgatgcacgaggccctgcacaatcactacacccagaagtccctgtctctgtcccctggcaaataa

SEQ ID NO: 367 - DNA, 1359 bp, synthetic construct
  source 1..1359: mol_type = other DNA
gaagtgcaattggtggaaagcggcggcggcctggtgcagccgggcggcagcctgcgcctgagctgcgcggcgtccggattcaacttttctgactactctatgagctgggtgcgccaggcaccgggcaaaggcctcgaatgggtgagccgtattaaagcttcttctggtggttctgactatgcggatagcgtgaaaggccgctttaccattagccgcgataattcgaaaaacaccctgtatctgcaaatgaacagcctgcgtgcggaagatactgcagtgtattattgcgcgcgtcagactgaagaccgttcttacggttacgacctggattattggggccaaggcaccctggtgacggtgagcagcgcctctaccaagggcccctctgtgtttcctctggctccctccagcaagtctacctctggtggaacagctgccctgggctgcctggtcaaggattactttcctgagcctgtcaccgtgtcctggaactctggcgctctgacatctggcgtgcacacctttccagctgtgctccagtcctccggcctgtactctctgtcctctgtcgtgaccgtgccttctagctctctgggcacccagacctacatctgcaatgtgaaccacaagccttccaacaccaaggtggacaagaaggtggaacccaagtcctgcgacaagacccacacctgtcctccatgtcctgctccagaactgctcggcggaccttccgtgttcctgtttcctccaaagcctaaggacaccctgatgatctctcggacccctgaagtgacctgcgtggtggtggatgtgtctcacgaagatcccgaagtgaagttcaactggtacgtggacggcgtggaagtgcacaacgccaagaccaagcctagagaggaacagtacaactccacctacagagtggtgtccgtgctgaccgtgctgcaccaggattggctgaacggcaaagagtacaagtgcaaggtgtccaacaaggccctgcctgctcctatcgaaaagaccatctccaaggccaagggccagcctagggaaccccaggtttacaccttgcctccatctcgggacgagctgaccaagaaccaggtgtccctgacctgtctcgtgaagggcttctacccctccgacatcgccgtggaatgggagtctaatggccagcctgagaacaactacaagacaacccctcctgtgctggactccgacggctcattcttcctgtactccaagctgacagtggacaagtccagatggcagcagggcaacgtgttctcctgctccgtgatgcacgaggccctgcacaatcactacacccagaagtccctgtctctgtcccctggcaaataa

SEQ ID NO: 368 - protein, 17 aa, synthetic construct
  UNSURE 1: note = G, A, V, L, I, S, T, C, M, N, Q, K, R, D, E, F, Y, H, P or W
  UNSURE 3..10: note = G, A, V, L, I, S, T, C, M, N, Q, K, R, D, E, F, Y, H, P or W
XIXXXXXXXXYADSVKG